European Patent Application EP 4 487 854 A1, published January 8, 2025. Title: 線維化疾患の治療又は予防のための医薬組成物. Applicant: 国立大学法人九州大学. The sequence listing filed with the application follows.

SEQUENCE LISTING (15 sequences)

SEQ ID NO: 1 - DNA, 21 bp, synthetic construct
  source 1..21: mol_type = other DNA
  misc_feature 1..19: note = RNA
  misc_feature 20..21: note = DNA
  misc_feature 1..21: note = sense strand of mouse si P4HA3 #1
ccacgagtatggacaggaatt

SEQ ID NO: 2 - DNA, 21 bp, synthetic construct
  source 1..21: mol_type = other DNA
  misc_feature 1..19: note = RNA
  misc_feature 20..21: note = DNA
  misc_feature 1..21: note = antisense strand of mouse si P4HA3 #1
ttcctgtccatactcgtggat

SEQ ID NO: 3 - DNA, 21 bp, synthetic construct
  source 1..21: mol_type = other DNA
  misc_feature 1..19: note = RNA
  misc_feature 20..21: note = DNA
  misc_feature 1..21: note = antisense strand of mouse si P4HA3 #1
gctcatagctctctaccattt

SEQ ID NO: 4 - DNA, 21 bp, synthetic construct
  source 1..21: mol_type = other DNA
  misc_feature 1..19: note = RNA
  misc_feature 20..21: note = DNA
  misc_feature 1..21: note = antisense strand of mouse si P4HA3 #1
atggtagagagctatgagcgg

SEQ ID NO: 5 - RNA, 19 nt, synthetic construct
  source 1..19: mol_type = other RNA
  misc_feature 1..19: note = partial sequence of SEQ ID NO.:1 which is fully complementary to SEQ ID NO.:2
ccacgagtatggacaggaa

SEQ ID NO: 6 - RNA, 19 nt, synthetic construct
  source 1..19: mol_type = other RNA
  misc_feature 1..19: note = partial sequence of SEQ ID NO.:2 which is fully complementary to SEQ ID NO.:1
ttcctgtccatactcgtgg

SEQ ID NO: 7 - RNA, 19 nt, synthetic construct
  source 1..19: mol_type = other RNA
  misc_feature 1..19: note = partial sequence of SEQ ID NO.:3 which is fully complementary to SEQ ID NO.:4
gctcatagctctctaccat

SEQ ID NO: 8 - RNA, 19 nt, synthetic construct
  source 1..19: mol_type = other RNA
  misc_feature 1..19: note = partial sequence of SEQ ID NO.:4 which is fully complementary to SEQ ID NO.:3
atggtagagagctatgagc

SEQ ID NO: 9 - DNA, 2255 bp, Homo sapiens
  source 1..2255: mol_type = other DNA
  misc_feature 1..2255: note = prolyl 4-hydroxylase subunit alpha 3 (P4HA3), transcript variant 1
gtctgaggggaagttcgcgagcgctggctatgggtcctggggcgcggctggcggcgctgctggcggtgctggcgctcgggacaggagacccagaaagggctgcggctcggggcgacacgttctcggcgctgaccagcgtggcgcgcgccctggcgcccgagcgccggctgctggggctgctgaggcggtacctgcgcggggaggaggcgcggctgcgggacctgactagattctacgacaaggtactttctttgcatgaggattcaacaacccctgtggctaaccctctgcttgcatttactctcatcaaacgcctgcagtctgactggaggaatgtggtacatagtctggaggccagtgagaacatccgagctctgaaggatggctatgagaaggtggagcaagaccttccagcctttgaggaccttgagggagcagcaagggccctgatgcggctgcaggacgtgtacatgctcaatgtgaaaggcctggcccgaggtgtctttcagagagtcactggctctgccatcactgacctgtacagccccaaacggctcttttctctcacaggggatgactgcttccaagttggcaaggtggcctatgacatgggggattattaccatgccattccatggctggaggaggctgtcagtctcttccgaggatcttacggagagtggaagacagaggatgaggcaagtctagaagatgccttggatcacttggcctttgcttatttccgggcaggaaatgtttcgtgtgccctcagcctctctcgggagtttcttctctacagcccagataataagaggatggccaggaatgtcttgaaatatgaaaggctcttggcagagagccccaaccacgtggtagctgaggctgtcatccagaggcccaatataccccacctgcagaccagagacacctacgaggggctatgtcagaccctgggttcccagcccactctctaccagatccctagcctctactgttcctatgagaccaattccaacgcctacctgctgctccagcccatccggaaggaggtcatccacctggagccctacattgctctctaccatgacttcgtcagtgactcagaggctcagaaaattagagaacttgcagaaccatggctacagaggtcagtggtggcatcaggggagaagcagttacaagtggagtaccgcatcagcaaaagtgcctggctgaaggacactgttgacccaaaactggtgaccctcaaccaccgcattgctgccctcacaggccttgatgtccggcctccctatgcagagtatctgcaggtggtgaactatggcatcggaggacactatgagcctcactttgaccatgctacgtcaccaagcagccccctctacagaatgaagtcaggaaaccgagttgcaacatttatgatctatctgagctcggtggaagctggaggagccacagccttcatctatgccaacctcagcgtgcctgtggttaggaatgcagcactgttttggtggaacctgcacaggagtggtgaaggggacagtgacacacttcatgctggctgtcctgtcctggtgggagataagtgggtggccaacaagtggatacatgagtatggacaggaattccgcagaccctgcagctccagccctgaagactgaactgttggcagagagaagctggtggagtcctgtggctttccagagaagccaggagccaaaagctggggtaggagaggagaaagcagagcagcctcctggaagaaggccttgtcagctttgtctgtgcctcgcaaatcagaggcaagggagaggttgttaccaggggacactgagaatgtacatttgatctgccccagccacggaagtcagagtaggatgcacagtacaaaggaggggggagtggaggcctgagagggaagtttctggagttcagatactctctgttgggaacaggacatctcaacagtctcaggttcgatcagtgggtcttttggcactttgaaccttgaccacagggaccaagaagtggcaatgaggacacctgcaggaggggctagcctgactcccagaactttaagactttctccccactgccttctgctgcagcccaagcagggagtgtccccctcccagaagcatatcccagatgagtggtacattatataaggattttttttaagttgaaaacaactttcttttctttttgtatgatggttttttaacacagtcattaaaaatgtttataaatca

SEQ ID NO: 10 - DNA, 2248 bp, Homo sapiens
  source 1..2248: mol_type = other DNA
  misc_feature 1..2248: note = prolyl 4-hydroxylase subunit alpha 3 (P4HA3), transcript variant 2
gtctgaggggaagttcgcgagcgctggctatgggtcctggggcgcggctggcggcgctgctggcggtgctggcgctcgggacaggagacccagaaagggctgcggctcggggcgacacgttctcggcgctgaccagcgtggcgcgcgccctggcgcccgagcgccggctgctggggctgctgaggcggtacctgcgcggggaggaggcgcggctgcgggacctgactagattctacgacaaggtactttctttgcatgaggattcaacaacccctgtggctaaccctctgcttgcatttactctcatcaaacgcctgcagtctgactggaggaatgtggtacatagtctggaggccagtgagaacatccgagctctgaaggatggctatgagaaggtggagcaagaccttccagcctttgaggaccttgagggagcagcaagggccctgatgcggctgcaggacgtgtacatgctcaatgtgaaaggcctggcccgaggtgtctttcagagagtcactggctctgccatcactgacctgtacagccccaaacggctcttttctctcacaggggatgactgcttccaagttggcaaggtggcctatgacatgggggattattaccatgccattccatggctggaggaggctgtcagtctcttccgaggatcttacggagagtggaagacagaggatgaggcaagtctagaagatgccttggatcacttggcctttgcttatttccgggcaggaaatgtttcgtgtgccctcagcctctctcgggagtttcttctctacagcccagataataagaggatggccaggaatgtcttgaaatatgaaaggctcttggcagagagccccaaccacgtggtagctgaggctgtcatccagaggcccaatataccccacctgcagaccagagacacctacgaggggctatgtcagaccctgggttcccagcccactctctaccagatccctagcctctactgttcctatgagaccaattccaacgcctacctgctgctccagcccatccggaaggaggtcatccacctggagccctacattgctctctaccatgacttcgtcagtgactcagaggctcagaaaattagagaacttgcagaaccatggctacagaggtcagtggtggcatcaggggagaagcagttacaagtggagtaccgcatcagcaaaagtgcctggctgaaggacactgttgacccaaaactggtgaccctcaaccaccgcattgctgccctcacaggccttgatgtccggcctccctatgcagagtatctgcaggtggtgaactatggcatcggaggacactatgagcctcactttgaccatgctacgtcaccaagcagccccctctacagaatgaagtcaggaaaccgagttgcaacatttatgatctatctgagctcggtggaagctggaggagccacagccttcatctatgccaacctcagcgtgcctgtggttaggcactgttttggtggaacctgcacaggagtggtgaaggggacagtgacacacttcatgctggctgtcctgtcctggtgggagataagtgggtggccaacaagtggatacatgagtatggacaggaattccgcagaccctgcagctccagccctgaagactgaactgttggcagagagaagctggtggagtcctgtggctttccagagaagccaggagccaaaagctggggtaggagaggagaaagcagagcagcctcctggaagaaggccttgtcagctttgtctgtgcctcgcaaatcagaggcaagggagaggttgttaccaggggacactgagaatgtacatttgatctgccccagccacggaagtcagagtaggatgcacagtacaaaggaggggggagtggaggcctgagagggaagtttctggagttcagatactctctgttgggaacaggacatctcaacagtctcaggttcgatcagtgggtcttttggcactttgaaccttgaccacagggaccaagaagtggcaatgaggacacctgcaggaggggctagcctgactcccagaactttaagactttctccccactgccttctgctgcagcccaagcagggagtgtccccctcccagaagcatatcccagatgagtggtacattatataaggattttttttaagttgaaaacaactttcttttctttttgtatgatggttttttaacacagtcattaaaaatgtttataaatca

SEQ ID NO: 11 - DNA, 2361 bp, Mus musculus
  source 1..2361: mol_type = other DNA
  misc_feature 1..2361: note = procollagen-proline, 2-oxoglutarate 4-dioxygenase (proline 4-hydroxylase),alpha polypeptide III (P4ha3)
gcgcgaccctgcgatgggcccaggggcgcggctggctctgctggcgctgctggcgctcgggggagaccccgcggcggccacggggcgggaggacacgttctccgcgctgaccagcgtggcgcgcgccctggcgcccgagcgcaggctgctggggacactgaggcgctacctgcgcggcgaggaggcgcggctgcgcgacttgaccagattctatgacaaggtactttctttgcacgaggacttgaagatccctgtagtgaatcctctacttgccttcactctcatcaaacgtctgcagtccgactggaggaatgtggtacatagtctggaggccactgagaacatccgagctctgaaggatggctatgagaaggtagagcaagaccttcctgcctttgaggacctcgagggagcagcaagggccctgatgcggctgcaggatgtgtacatgctcaacgtgaagggcttggctcgaggcgtcttccagagggtcacgggctcctccatcaccgacctgtacagtcccaggcagctcttctctctcacagcggatgactgcttccaagttggcaaggtggcctatgacacaggggattactaccatgccatcccatggctggaggaagctgtcagtctcttccggagagcccacggcgagtggaagacagaggacgaggccagtctggaagacgccctggattacttggcctttgcctgtttccaggtaggaaatgtttcatgtgccctcagcctctctcgagagttccttgtctacagcccagacaataagaggatggccaggaatgtgttgaaatatgaaaggctcttggctgagaatggtcaccagatggcggctgagactgcaattcagaggcccaacgtaccccacctgcagaccagggacacctacgaggggctatgccagaccctgggctcccagccaacacactaccaaatccccagcctctactgctcctatgagaccaattccagcccctacctactgctccagcctgcccgaaaggaggttgtccacctacggccgctcatagctctctaccatgactttgtcagtgacgaggaagctcagaaaatccgagagcttgcagaaccgtggctccagagatcagtggtggcttcgggggaaaagcagttgcaagtggagtaccgcatcagcaaaagtgcctggctaaaggacacggttgatccaatgctggtgacccttgaccaccgcattgcggccctcacaggccttgacatccagcctccctacgcagagtatctccaggtggtgaactatggaatcggagggcactatgagcctcactttgaccatgctacgtcgcccagcagccccctgtacagaatgaagtctgggaaccgagtggcaacgtttatgatctatctgagctccgtagaagctggaggagccacggcttttatctatggcaacttcagtgtgcctgtggttaagaatgctgcactgttttggtggaacctgcacaggagcggagagggggatggtgacacacttcatgctggctgtcctgtgctggtgggagacaagtgggtggccaacaagtggatccacgagtatggacaggaattccgaagaccctgcagcaccaaccctgaagactgaaacactggcagatggcagcttgtcagagaagccaggagccaaagccatgggcagaggggagccgaccctcctgaaggaaggcctccagcaaggctgctgcctgtgagtcaaggataggactttactaggaagccccctatcccccaaatttgcatctgtttctactccagctgtgagacttaagagtcgaatggacaagacgaagaggcctaagagggcgcagatgtccttaggaataaaaggattgagctcagtgtagaaactcagggtttagaatgtgcctgggtttagttcactaacactgaacacacaccacatacacacacacacacacacacacacacacacacacacacacacacatatccatacacccatccacatatacccatatacacacacatgcatacacacacacacacacacacccatacacccacatatacccatacacacagacatgcgtacacacatatacatacacatatatacaagcacacacacacacatccatacacccatcctcatatacccacacacacactgcaaacaataatggggctgatttctgctgctgccccaggaggagtgtctgacccagaggcctccatccccatccccagtggggatatcatgtgacgactgacttttaaagtggaaaacaattttgttttcctttttgtgatggtttttattgtcattaaaatgttttacaaaca

SEQ ID NO: 12 - DNA, 21 bp, synthetic construct
  source 1..21: mol_type = other DNA
  misc_feature 1..19: note = RNA
  misc_feature 20..21: note = DNA
  misc_feature 1..21: note = sense strand of mouse si Hsp47
cggacaggcctgtacaacttt

SEQ ID NO: 13 - DNA, 21 bp, synthetic construct
  source 1..21: mol_type = other DNA
  misc_feature 1..19: note = RNA
  misc_feature 20..21: note = DNA
  misc_feature 1..21: note = antisense strand of mouse si Hsp47
agttgtacaggcctgtccggt

SEQ ID NO: 14 - DNA, 21 bp, synthetic construct
  source 1..21: mol_type = other DNA
  misc_feature 1..19: note = RNA
  misc_feature 20..21: note = DNA
  misc_feature 1..21: note = sense strand of mouse si SMAD3
ggaatttgctgccctcctatt

SEQ ID NO: 15 - DNA, 21 bp, synthetic construct
  source 1..21: mol_type = other DNA
  misc_feature 1..19: note = RNA
  misc_feature 20..21: note = DNA
  misc_feature 1..21: note = antisense strand of mouse si SMAD3
taggagggcagcaaattccct